European Patent Specification EP 3 426 759 B1, published July 26, 2023. Title: Particles Including Enzyme. Applicant: The Procter & Gamble Company. The sequence listing filed with the application follows.

SEQUENCE LISTING (6 sequences)

SEQ ID NO: 1 - protein, 109 aa, Bacillus licheniformis
ARYDDVLYFPASRYPETGAHISDAIKAGHADVCTIERSGADKRRQESLKGIPTKPGFDRDEWPMAMCEEGGKGASVRYVSSSDNRGAGSWVGNRLNGYADGTRILFIVQ

SEQ ID NO: 2 - protein, 109 aa, Bacillus subtilis
ASSYDKVLYFPLSRYPETGSHIRDAIAEGHPDICTIDDGADKRREESLKGIPTKPGYDRDEWPMAVCEEGGAGADVRYVTPSDNRGAGSWVGNQMSSYPDGTRVLFIVQ

SEQ ID NO: 3 - protein, 109 aa, Bacillus licheniformis
ARYDDILYFPASRYPETGAHISDAIKAGHSDVCTIERSGADKRRQESLKGIPTKPGFDRDEWPMAMCEEGGKGASVRYVSSSDNRGAGSWVGNRLSGFADGTRILFIVQ

SEQ ID NO: 4 - protein, 361 aa, Aggregatibacter actinomycetemcomitans
NCCVKGNSIYPQKTSTKQTGLMLDIARHFYSPEVIKSFIDTISLSGGNFLHLHFSDHENYAIESHLLNQRAENAVQGKDGIYINPYTGKPFLSYRQLDDIKAYAKAKGIELIPELDSPNHMTAIFKLVQKDRGVKYLQGLKSRQVDDEIDITNADSITFMQSLMSEVIDIFGDTSQHFHIGGDEFGYSVESNHEFITYANKLSYFLEKKGLKTRMWNDGLIKNTFEQINPNIEITYWSYDGDTQDKNEAAERRDMRVSLPELLAKGFTVLNYNSYYLYIVPKASPTFSQDAAFAAKDVIKNWDLGVWDGRNTKNRVQNTHEIAGAALSIWGEDAKALKDETIQKNTKSLLEAVIHKTNGDE

SEQ ID NO: 5 - protein, 204 aa, Aspergillus oryzae
KTGSGDSQSDPIKADLEVKGQSALPFDVDCWAILCKGAPNVLQRVNEKTKNSNRDRSGANKGPFKDPQKWGIKALPPKNPSWSAQDFKSPEEYAFASSLQGGTNAILAPVNLASQNSQGGVLNGFYSANKVAQFDPSKPQQTKGTWFQITKFTGAAGPYCKALGSNDKSVCDKNKNIAGDWGFDPAKWAYQYDEKNNKFNYVGK

SEQ ID NO: 6 - protein, 188 aa, Trichoderma harzianum
APAPMPTPPGIPTESSARTQLAGLTVAVAGSGTGYSRDLFPTWDAISGNCNAREYVLKRDGEGVQVNNACESQSGTWISPYDNASFTNASSLDIDHMVPLKNAWISGASSWTTAQREALANDVSRPQLWAVSASANRSKGDRSPDQWKPPLTSFYCTYAKSWIDVKSFYKLTITSAEKTALSSMLDTC